European Patent Application EP 4 368 703 A1, published May 15, 2024. Title: Oxidative Stress Resistant Mesenchymal Stem Cell, Preparation Method Thereof and Its Use. Applicant: TOOLGEN INCORPORATED. Application KR PCT220305, filed July 8, 2022. The sequence listing filed with the application follows.

SEQUENCE LISTING (61 sequences)

SEQ ID NO: 1 - DNA, 23 bp, Homo sapiens
  source 1..23: mol_type = genomic DNA
tgcagtcacagtgccctgagggg

SEQ ID NO: 2 - DNA, 23 bp, Homo sapiens
  source 1..23: mol_type = genomic DNA
gaaggtgcggttgccatgctggg

SEQ ID NO: 3 - DNA, 23 bp, Homo sapiens
  source 1..23: mol_type = genomic DNA
tgaaggtgcggttgccatgctgg

SEQ ID NO: 4 - DNA, 23 bp, Homo sapiens
  source 1..23: mol_type = genomic DNA
gatcataccaagcaggcctttgg

SEQ ID NO: 5 - DNA, 23 bp, Homo sapiens
  source 1..23: mol_type = genomic DNA
ttggcatcatgaacgagctgcgg

SEQ ID NO: 6 - DNA, 23 bp, Homo sapiens
  source 1..23: mol_type = genomic DNA
tgaggccagcaccaccttgtggg

SEQ ID NO: 7 - DNA, 23 bp, Homo sapiens
  source 1..23: mol_type = genomic DNA
catggccttgaagacagggctgg

SEQ ID NO: 8 - DNA, 23 bp, Homo sapiens
  source 1..23: mol_type = genomic DNA
gtgaacatggccttgaagacagg

SEQ ID NO: 9 - DNA, 23 bp, Homo sapiens
  source 1..23: mol_type = genomic DNA
ccatgttcaccaacgggctgcgg

SEQ ID NO: 10 - DNA, 23 bp, Homo sapiens
  source 1..23: mol_type = genomic DNA
atggaggtggtgtccattgaggg

SEQ ID NO: 11 - DNA, 23 bp, Homo sapiens
  source 1..23: mol_type = genomic DNA
ccaggtagctgagcgactgtcgg

SEQ ID NO: 12 - DNA, 23 bp, Homo sapiens
  source 1..23: mol_type = genomic DNA
gaggcttacaaccccagtgacgg

SEQ ID NO: 13 - DNA, 23 bp, Homo sapiens
  source 1..23: mol_type = genomic DNA
tcatggggttgtaacagtccagg

SEQ ID NO: 14 - DNA, 23 bp, Homo sapiens
  source 1..23: mol_type = genomic DNA
acaaccccatgaccaatcagtgg

SEQ ID NO: 15 - DNA, 23 bp, Homo sapiens
  source 1..23: mol_type = genomic DNA
ctgcatccaccacaacagtgtgg

SEQ ID NO: 16 - DNA, 23 bp, Homo sapiens
  source 1..23: mol_type = genomic DNA
gatgtgctcactgagtctgaagg

SEQ ID NO: 17 - DNA, 20 bp, synthetic construct
  source 1..20: mol_type = other DNA
agccagatcccaggcctagc

SEQ ID NO: 18 - DNA, 20 bp, synthetic construct
  source 1..20: mol_type = other DNA
ccggtgcatcctggtacttg

SEQ ID NO: 19 - DNA, 20 bp, synthetic construct
  source 1..20: mol_type = other DNA
ttggcatcatgaacgagctg

SEQ ID NO: 20 - DNA, 20 bp, synthetic construct
  source 1..20: mol_type = other DNA
acttctcgcccatggagatg

SEQ ID NO: 21 - DNA, 20 bp, synthetic construct
  source 1..20: mol_type = other DNA
tggcccacaaggtggtgctg

SEQ ID NO: 22 - DNA, 20 bp, synthetic construct
  source 1..20: mol_type = other DNA
ggacaacgctgtcgatctgg

SEQ ID NO: 23 - DNA, 20 bp, synthetic construct
  source 1..20: mol_type = other DNA
cctggtcaagatcttcgagg

SEQ ID NO: 24 - DNA, 20 bp, synthetic construct
  source 1..20: mol_type = other DNA
gagttgttcctgccgcccac

SEQ ID NO: 25 - DNA, 20 bp, synthetic construct
  source 1..20: mol_type = other DNA
gtgggcggcaggaacaactc

SEQ ID NO: 26 - DNA, 20 bp, synthetic construct
  source 1..20: mol_type = other DNA
tccctgaagacaggaagagg

SEQ ID NO: 27 - DNA, 20 bp, synthetic construct
  source 1..20: mol_type = other DNA
acatgagctctctccttcct

SEQ ID NO: 28 - DNA, 22 bp, synthetic construct
  source 1..22: mol_type = other DNA
gggagaaattcacctgtctctt

SEQ ID NO: 29 - DNA, 25 bp, synthetic construct
  source 1..25: mol_type = other DNA
caagtgattagaatggatggctatg

SEQ ID NO: 30 - DNA, 21 bp, synthetic construct
  source 1..21: mol_type = other DNA
ggaaggagagagctcatgttt

SEQ ID NO: 31 - DNA, 24 bp, synthetic construct
  source 1..24: mol_type = other DNA
caactagatgaagagacaggtgaa

SEQ ID NO: 32 - DNA, 21 bp, synthetic construct
  source 1..21: mol_type = other DNA
gaggctgaggttggaaagtag

SEQ ID NO: 33 - DNA, 53 bp, synthetic construct
  source 1..53: mol_type = other DNA
acactctttccctacacgacgctcttccgatctgactacagtagttaatcatc

SEQ ID NO: 34 - DNA, 54 bp, synthetic construct
  source 1..54: mol_type = other DNA
gtgactggagttcagacgtgtgctcttccgatctcagatacaaaaagggttctc

SEQ ID NO: 35 - DNA, 22 bp, synthetic construct
  source 1..22: mol_type = other DNA
cctcaatcgtctcctttatgcc

SEQ ID NO: 36 - DNA, 20 bp, synthetic construct
  source 1..20: mol_type = other DNA
gatcattcgccactcgttcc

SEQ ID NO: 37 - DNA, 23 bp, synthetic construct
  source 1..23: mol_type = other DNA
cacatccagtcagaaaccagtgg

SEQ ID NO: 38 - DNA, 22 bp, synthetic construct
  source 1..22: mol_type = other DNA
ggaatgtctgcgccaaaagctg

SEQ ID NO: 39 - DNA, 23 bp, Homo sapiens
  source 1..23: mol_type = other DNA
atttgattgacatactttggagg

SEQ ID NO: 40 - DNA, 23 bp, Homo sapiens
  source 1..23: mol_type = genomic DNA
tggaggcaagatatagatcttgg

SEQ ID NO: 41 - DNA, 23 bp, Homo sapiens
  source 1..23: mol_type = genomic DNA
tatttgacttcagtcagcgacgg

SEQ ID NO: 42 - DNA, 23 bp, Homo sapiens
  source 1..23: mol_type = genomic DNA
gcgacggaaagagtatgagctgg

SEQ ID NO: 43 - DNA, 23 bp, Homo sapiens
  source 1..23: mol_type = genomic DNA
cactgttgatggtgggaagtggg

SEQ ID NO: 44 - DNA, 23 bp, Homo sapiens
  source 1..23: mol_type = genomic DNA
attatgccactgttgatggtggg

SEQ ID NO: 45 - DNA, 23 bp, Homo sapiens
  source 1..23: mol_type = genomic DNA
cattatgccactgttgatggtgg

SEQ ID NO: 46 - DNA, 23 bp, Homo sapiens
  source 1..23: mol_type = genomic DNA
gtacagagtactcagttcttggg

SEQ ID NO: 47 - DNA, 23 bp, Homo sapiens
  source 1..23: mol_type = genomic DNA
gttcttgggaaagttatggcagg

SEQ ID NO: 48 - DNA, 23 bp, Homo sapiens
  source 1..23: mol_type = genomic DNA
ggaaagttatggcaggtttaagg

SEQ ID NO: 49 - DNA, 23 bp, Homo sapiens
  source 1..23: mol_type = genomic DNA
gtacgcctccactgagtgcaagg

SEQ ID NO: 50 - DNA, 23 bp, Homo sapiens
  source 1..23: mol_type = genomic DNA
acagcgacggttctacgtccagg

SEQ ID NO: 51 - DNA, 23 bp, Homo sapiens
  source 1..23: mol_type = genomic DNA
gcagtccgactcccgctgcaagg

SEQ ID NO: 52 - DNA, 23 bp, Homo sapiens
  source 1..23: mol_type = genomic DNA
ctgtcggaagtagccgcccgcgg

SEQ ID NO: 53 - DNA, 23 bp, Homo sapiens
  source 1..23: mol_type = genomic DNA
ctgtcggaagtagccgcccgggg

SEQ ID NO: 54 - DNA, 23 bp, Homo sapiens
  source 1..23: mol_type = genomic DNA
gttacggggcacgctcatggggg

SEQ ID NO: 55 - DNA, 23 bp, Homo sapiens
  source 1..23: mol_type = genomic DNA
cgtgccccgtaaccgcatcgggg

SEQ ID NO: 56 - DNA, 23 bp, Homo sapiens
  source 1..23: mol_type = genomic DNA
cccaccccgatgcggttacgggg

SEQ ID NO: 57 - DNA, 20 bp, synthetic construct
  source 1..20: mol_type = other DNA
ctgaacgtgcgctgcgagtc

SEQ ID NO: 58 - DNA, 20 bp, synthetic construct
  source 1..20: mol_type = other DNA
agatcaggcggcccaccttg

SEQ ID NO: 59 - DNA, 20 bp, synthetic construct
  source 1..20: mol_type = other DNA
gacagtcgctcagctacctg

SEQ ID NO: 60 - DNA, 20 bp, synthetic construct
  source 1..20: mol_type = other DNA
gcgaccactgattggtcatg

SEQ ID NO: 61 - DNA, 20 bp, synthetic construct
  source 1..20: mol_type = other DNA
ctcagtgtcttgggacttgc